European Patent Application EP 4 242 314 A1, published September 13, 2023. Title: A Salmonella strain and use thereof for the prevention and treatment of cancer. Applicant: Industry Foundation of Chonnam National University. The sequence listing filed with the application follows.

SEQUENCE LISTING (17 sequences)

SEQ ID NO: 1 - protein, 305 aa, Artificial Sequence
  ClyA
MIMTGIFAEQTVEVVKSAIETADGALDLYNKYLDQVIPWKTFDETIKELSRFKQEYSQEASVLVGDIKVLLMDSQDKYFEATQTVYEWCGVVTQLLSAYILLFDEYNEKKASAQKDILIRILDDGVKKLNEAQKSLLTSSQSFNNASGKLLALDSQLTNDFSEKSSYFQSQVDRIRKEAYAGAAAGIVAGPFGLIISYSIAAGVIEGKLIPELNNRLKTVQNFFTSLSATVKQANKDIDAAKLKLATEIAAIGEIKTETETTRFYVDYDDLMLSLLKGAAKKMINTCNEYQQRHGKKTLFEVPDV

SEQ ID NO: 2 - DNA, 46 bp, Artificial Sequence
  Forward primer
cggaattcaccatgtctagattagataaaagtaaagtgattaacag

SEQ ID NO: 3 - DNA, 48 bp, Artificial Sequence
  Reverse primer
gctctagacagctgttaagacccactttcacatttaagttgtttttct

SEQ ID NO: 4 - DNA, 39 bp, Artificial Sequence
  Forward primer
ctactccgtcaagccgtcaagctgttgtgaccgcttgct

SEQ ID NO: 5 - DNA, 57 bp, Artificial Sequence
  Reverse primer
tgaattcctcctgctagctagttggtaacgaatcagacgccgggtaataccggatag

SEQ ID NO: 6 - DNA, 39 bp, Artificial Sequence
  Forward primer
tgctactccgtcaagccgtcaagctgttgtgaccgcttg

SEQ ID NO: 7 - DNA, 39 bp, Artificial Sequence
  Reverse primer
agcttggtaacgaatcagacgccgggtaataccggatag

SEQ ID NO: 8 - DNA, 6 bp, Artificial Sequence
  -35 promoter sequence
ttcgcg

SEQ ID NO: 9 - DNA, 9 bp, Artificial Sequence
  -10 promoter sequence
atgcataat

SEQ ID NO: 10 - DNA, 78 bp, Artificial Sequence
  Forward primer
ccctatgctactccgtcaagccgtcaattgttgacaattaatcatcggctcgtataatgtctgattcgttaccaagct

SEQ ID NO: 11 - DNA, 78 bp, Artificial Sequence
  Reverse primer
agcttggtaacgaatcagacattatacgagccgatgattaattgtcaacaattgacggcttgacggagtagcataggg

SEQ ID NO: 12 - DNA, 75 bp, Artificial Sequence
  Forward primer
tgctactccgtcaagccgtctttacagctagctcagtcctaggtataatgctagccaattgtctgattcgttacc

SEQ ID NO: 13 - DNA, 75 bp, Artificial Sequence
  Reverse primer
ggtaacgaatcagacaattggctagcattatacctaggactgagctagctgtaaagacggcttgacggagtagca

SEQ ID NO: 14 - DNA, 75 bp, Artificial Sequence
  Forward primer
tgctactccgtcaagccgtcttgacagctagctcagtcctaggtataatgctagccaattgtctgattcgttacc

SEQ ID NO: 15 - DNA, 75 bp, Artificial Sequence
  Reverse primer
ggtaacgaatcagacaattggctagcattatacctaggactgagctagctgtcaagacggcttgacggagtagca

SEQ ID NO: 16 - DNA, 192 bp, Unknown
  OXB1 promoter
aagctgttgtgaccgcttgctctagccagctatcgagttgtgaaccgatccatctagcaattggtctcgatctagcgataggcttcgatctagctatgtagaaacgccgtgtgctcgatcgcctgacgctttttatcgcaactctctactgttgcttcaacagaacatattgactatccggtattacccggc

SEQ ID NO: 17 - protein, 376 aa, Artificial Sequence
  FlaA
MAINVSTNVSAMTAQRYLNNAADGTQKSMERLSSGYKINSARDDAAGLQISNRLTSQSRGLDMAVRNANDGISIAQTAEGAMNETTNILQRMRDLSLQSANGSNSSSERQAIQEEVSALNDELNRIAETTSFGGNKLLNGSFGNKSFQIGADSGEAVMLSMSDMRSDTKAMGGKSYVATNGKAPDWSVTNATDLTLSYTDKQGEAREVTINAKAGDDLEEVATYINGQNGDIKASVGDEGKLQLFAANQKVSSDVTIGGGLGTEIGFAAGKDVTVKDINVTTVGGSQEAVALIDGALKAVDSQRASLGAFQNRFGHAISNLDNINENVNASRSRIKDTDYARETTQMTKSQILQQASTSVLAQAKQSPSAALSLLG